European Patent Application EP 4 159 864 A1, published April 5, 2023. Title: RECOMBINANT EXPRESSION VECTOR FOR PRODUCTION OF ENCAPSULIN-BASED VACCINE AND METHOD FOR MANUFACTURING THE SAME. Applicant: InThera Inc. The sequence listing filed with the application follows.

SEQUENCE LISTING (21 sequences)

SEQ ID NO: 1 - protein, 265 aa, Artificial Sequence [sequence omitted]

SEQ ID NO: 2 - protein, 159 aa, Artificial Sequence
  Rotavirus G1P[8] VP8* Human rotavirus A strain Wa
LDGPYQPTTFTPPTDYWILINSNTNGVVYESTNNSDFWTAVIAVEPHVNPVDRQYNVFGENKQFNVRNDSDKWKFLEMFRGSSQNDFYNRRTLTSDTRLVGILKYGGRIWTFHGETPRATTDSSNTANLNGISITIHSEFYIIPRSQESKCNEYINNGL

SEQ ID NO: 3 - protein, 160 aa, Artificial Sequence
  Rotavirus 1076 G2P[6] isolate RVA/Human/Sweden/1076/1983/G2P2A[6]
VLDGPYQPTSFKPPSDYWILLNPTNQQVVLEGTNKTDIWVALLLVEPNVTNQSRQYTLFGETKQITVENNTNKWKFFEMFRSSVSAEFQHKRTLTSDTKLAGFLKFYNSVWTFYGETPHATTDYSSTSNLSEVETAIHVEFYIIPRSQESKCNEYINTGL

SEQ ID NO: 4 - protein, 160 aa, Artificial Sequence
  Rotavirus DS-1 G2P[4] isolate RVA/Human/Sweden/1076/1983/G2P2A[6]
VLDGPYQPTTFKPPNDYWLLISSNTNGVVYESTNNNDFWTAVIAVEPHVSQTNRQYILFGENKQFNVENNSDKWKFFEMFKGSSQGDFSNRRTLTSSNRLVGMLKYGGRVWTFHGETPRATTDSSNTADLNNISIIIHSEFYIIPRSQESKCNEYINNGL

SEQ ID NO: 5 - protein, 101 aa, Artificial Sequence
  Dengue Virus Type 1 EDIII (EF654110.1)
KGVSYVMCTGSFKLEKEVAETQHGTVLVQVKYEGTDAPCKIPFSSQDEKGVTQNGRLITANPIVTDKEKPVNIEAEPPFGESYLVVGAGEKALKLSWFKKG

SEQ ID NO: 6 - protein, 101 aa, Artificial Sequence
  Dengue Virus Type 2 EDIII (KP406804.1)
KGMSYSMCTGKFKVVKEIAETQHGTIVIRVQYEGDGSPCKIPFEIMDLEKRHVLGRLITVNPIVTEKDRPVNIEAEPPFGDSYIIIGVEPGQLKLNWFKKG

SEQ ID NO: 7 - protein, 101 aa, Artificial Sequence
  Dengue Virus Type 3 EDIII (KP406805.1)
KGMSYAMCLNTFVLKKEVSETQHGTILIKVEYKGKDAPCKIPFSTEDGQGKAHNGRLITANPVVTKEEEPVNIEAEPPFGESNIVIGIGDKALKINWYRKG

SEQ ID NO: 8 - protein, 101 aa, Artificial Sequence
  Dengue Virus Type 4 EDIII (KP406806.1)
KGMSYTMCSGKFSIDKEMAETQHGTTVVRVKYEGAGAPCKVPIEIRDVNKEKVVGRIISSTPFAEYTDSVTNIELEPPFGDSYIVIGVGDSALTLHWFRKG

SEQ ID NO: 9 - protein, 35 aa, Artificial Sequence
  HPV E7
GQAEPDRAHYNIVTFCCKCDSTLRLCVQSTHVDIR

SEQ ID NO: 10 - DNA, 669 bp, Artificial Sequence
  2019-nCoV RBD of spike S protein 319-541 (223a.a.)
cgcgtgcagccgactgaatctattgttcgcttcccgaacatcaccaacctgtgcccgttcggcgaagttttcaacgcaacccgtttcgctagcgtttacgcgtggaaccgtaaacgtatctccaactgcgttgctgattactctgttctgtataactctgcatctttcagcaccttcaaatgttacggcgtgagcccgaccaaactgaacgatctgtgcttcaccaacgtgtacgctgatagcttcgtgatccgtggcgatgaagttcgtcagatcgcgccgggtcagaccggtaaaattgctgactacaactacaaactgccggatgatttcaccggttgcgttatcgcgtggaactctaacaacctggattctaaagtgggcggtaactacaactacctgtaccgtctgttccgcaaatctaacctgaaaccgttcgaacgcgatatctccaccgaaatctaccaggcaggttctaccccgtgcaacggtgttgaaggtttcaactgctacttcccgctgcagtcctacggttttcagccgaccaacggtgttggttaccagccgtaccgcgttgtggtgctgtctttcgaactgctgcacgcgccggcgaccgtttgcggtccgaagaaaagcaccaacctggttaaaaacaaatgcgttaacttc

SEQ ID NO: 11 - DNA, 4341 bp, Artificial Sequence
  Vector Map (pET-9a)
ttctcatgtttgacagcttatcatcgataagctttaatgcggtagtttatcacagttaaattgctaacgcagtcaggcaccgtgtatgaaatctaacaatgcgctcatcgtcatcctcggcaccgtcaccctggatgctgtaggcataggcttggttatgccggtactgccgggcctcttgcgggatatcgtccattccgacagcatcgccagtcactatggcgtgctgctagcgctatatgcgttgatgcaatttctatgcgcacccgttctcggagcactgtccgaccgctttggccgccgcccagtcctgctcgcttcgctacttggagccactatcgactacgcgatcatggcgaccacacccgtcctgtggatatccggatatagttcctcctttcagcaaaaaacccctcaagacccgtttagaggccccaaggggttatgctagttattgctcagcggtggcagcagccaactcagcttcctttcgggctttgttagcagccggatccgcgacccatttgctgtccaccagtcatgctagccatatgtatatctccttcttaaagttaaacaaaattatttctagagggaaaccgttgtggtctccctatagtgagtcgtattaatttcgcgggatcgagatctcgatcctctacgccggacgcatcgtggccggcatcaccggcgccacaggtgcggttgctggcgcctatatcgccgacatcaccgatggggaagatcgggctcgccacttcgggctcatgagcgcttgtttcggcgtgggtatggtggcaggccccgtggccgggggactgttgggcgccatctccttgcatgcaccattccttgcggcggcggtgctcaacggcctcaacctactactgggctgcttcctaatgcaggagtcgcataagggagagcgtcgaccgatgcccttgagagccttcaacccagtcagctccttccggtgggcgcggggcatgactatcgtcgccgcacttatgactgtcttctttatcatgcaactcgtaggacaggtgccggcagcgctctgggtcattttcggcgaggaccgctttcgctggagcgcgacgatgatcggcctgtcgcttgcggtattcggaatcttgcacgccctcgctcaagccttcgtcactggtcccgccaccaaacgtttcggcgagaagcaggccattatcgccggcatggcggccgacgcgctgggctacgtcttgctggcgttcgcgacgcgaggctggatggccttccccattatgattcttctcgcttccggcggcatcgggatgcccgcgttgcaggccatgctgtccaggcaggtagatgacgaccatcagggacagcttcaaggatcgctcgcggctcttaccagcctaacttcgatcactggaccgctgatcgtcacggcgatttatgccgcctcggcgagcacatggaacgggttggcatggattgtaggcgccgccctataccttgtctgcctccccgcgttgcgtcgcggtgcatggagccgggccacctcgacctgaatggaagccggcggcacctcgctaacggattcaccactccaagaattggagccaatcaattcttgcggagaactgtgaatgcgcaaaccaacccttggcagaacatatccatcgcgtccgccatctccagcagccgcacgcggcgcatctcgggcagcgttgggtcctggccacgggtgcgcatgatcgtgctcctgtcgttgaggacccggctaggctggcggggttgccttactggttagcagaatgaatcaccgatacgcgagcgaacgtgaagcgactgctgctgcaaaacgtctgcgacctgagcaacaacatgaatggtcttcggtttccgtgtttcgtaaagtctggaaacgcggaagtcagcgccctgcaccattatgttccggatctgcatcgcaggatgctgctggctaccctgtggaacacctacatctgtattaacgaagcgctggcattgaccctgagtgatttttctctggtcccgccgcatccataccgccagttgtttaccctcacaacgttccagtaaccgggcatgttcatcatcagtaacccgtatcgtgagcatcctctctcgtttcatcggtatcattacccccatgaacagaaatcccccttacacggaggcatcagtgaccaaacaggaaaaaaccgcccttaacatggcccgctttatcagaagccagacattaacgcttctggagaaactcaacgagctggacgcggatgaacaggcagacatctgtgaatcgcttcacgaccacgctgatgagctttaccgcagctgcctcgcgcgtttcggtgatgacggtgaaaacctctgacacatgcagctcccggagacggtcacagcttgtctgtaagcggatgccgggagcagacaagcccgtcagggcgcgtcagcgggtgttggcgggtgtcggggcgcagccatgacccagtcacgtagcgatagcggagtgtatactggcttaactatgcggcatcagagcagattgtactgagagtgcaccatatatgcggtgtgaaataccgcacagatgcgtaaggagaaaataccgcatcaggcgctcttccgcttcctcgctcactgactcgctgcgctcggtcgttcggctgcggcgagcggtatcagctcactcaaaggcggtaatacggttatccacagaatcaggggataacgcaggaaagaacatgtgagcaaaaggccagcaaaaggccaggaaccgtaaaaaggccgcgttgctggcgtttttccataggctccgcccccctgacgagcatcacaaaaatcgacgctcaagtcagaggtggcgaaacccgacaggactataaagataccaggcgtttccccctggaagctccctcgtgcgctctcctgttccgaccctgccgcttaccggatacctgtccgcctttctcccttcgggaagcgtggcgctttctcatagctcacgctgtaggtatctcagttcggtgtaggtcgttcgctccaagctgggctgtgtgcacgaaccccccgttcagcccgaccgctgcgccttatccggtaactatcgtcttgagtccaacccggtaagacacgacttatcgccactggcagcagccactggtaacaggattagcagagcgaggtatgtaggcggtgctacagagttcttgaagtggtggcctaactacggctacactagaaggacagtatttggtatctgcgctctgctgaagccagttaccttcggaaaaagagttggtagctcttgatccggcaaacaaaccaccgctggtagcggtggtttttttgtttgcaagcagcagattacgcgcagaaaaaaaggatctcaagaagatcctttgatcttttctacggggtctgacgctcagtggaacgaaaactcacgttaagggattttggtcatgaacaataaaactgtctgcttacataaacagtaatacaaggggtgttatgagccatattcaacgggaaacgtcttgctcgaggccgcgattaaattccaacatggatgctgatttatatgggtataaatgggctcgcgataatgtcgggcaatcaggtgcgacaatctatcgattgtatgggaagcccgatgcgccagagttgtttctgaaacatggcaaaggtagcgttgccaatgatgttacagatgagatggtcagactaaactggctgacggaatttatgcctcttccgaccatcaagcattttatccgtactcctgatgatgcatggttactcaccactgcgatccccgggaaaacagcattccaggtattagaagaatatcctgattcaggtgaaaatattgttgatgcgctggcagtgttcctgcgccggttgcattcgattcctgtttgtaattgtccttttaacagcgatcgcgtatttcgtctcgctcaggcgcaatcacgaatgaataacggtttggttgatgcgagtgattttgatgacgagcgtaatggctggcctgttgaacaagtctggaaagaaatgcataagcttttgccattctcaccggattcagtcgtcactcatggtgatttctcacttgataaccttatttttgacgaggggaaattaataggttgtattgatgttggacgagtcggaatcgcagaccgataccaggatcttgccatcctatggaactgcctcggtgagttttctccttcattacagaaacggctttttcaaaaatatggtattgataatcctgatatgaataaattgcagtttcatttgatgctcgatgagtttttctaagaa

SEQ ID NO: 12 - protein, 7 aa, Artificial Sequence
  MSAVKAA
MSAVKAA

SEQ ID NO: 13 - protein, 70 aa, Artificial Sequence
  ARSNTD
AAVQAAEVKVDGSEPKLSKNELKRRLKAEKKVAEKEAKQKELSEKQLSQATAAATNHTTDNGVGPEEESV

SEQ ID NO: 14 - protein, 70 aa, Artificial Sequence
  MARSNTD(9)
AAVQAAEVKVDGSEPKLSANELAARLAAEAAVAEAEAAQAELSEKQLSQATAAATNHTTDNGVGPEEESV

SEQ ID NO: 15 - DNA, 24 bp, Artificial Sequence
  LINKER1
ggcggtggctctggcggtggctct

SEQ ID NO: 16 - DNA, 18 bp, Artificial Sequence
  LINKER2
ggttctggttctggttct

SEQ ID NO: 17 - DNA, 54 bp, Artificial Sequence
  LINKER3-1
ggcggtggctctggcggtggctctcaccatcaccatcaccatggcggtggctct

SEQ ID NO: 18 - DNA, 39 bp, Artificial Sequence
  LINKER3-2
ggcggtggctctgaagcggccgcgaaaggcggtggctct

SEQ ID NO: 19 - DNA, 51 bp, Artificial Sequence
  LINKER3-3
ggcggtggctctggcggtggctctgaagcggccgcgaaaggcggtggctct

SEQ ID NO: 20 - DNA, 51 bp, Artificial Sequence
  Linker3-4
ggcggtgggagcggcggtggctctgaagcggccgcgaaaggcggtggctct

SEQ ID NO: 21 - protein, 6 aa, Artificial Sequence
  6xHIS tag
HHHHHH